European Patent Application EP 4 299 730 A1, published January 3, 2024. Title: METHOD OF MANUFACTURING FERMENTED FOOD/BEVERAGE, AND METHOD OF ANAEROBIC FERMENTATION. Applicant: Amano Enzyme Inc. KAMON, Masahiro TADA, Shusaku. The sequence listing filed with the application follows.

SEQUENCE LISTING (1 sequence)

SEQ ID NO: 1 - protein, 505 aa, Acremonium chrysogenum
MRSLAPLLSIAALARASPVDTSLLTRQETLNTCLEAAELSYVDVNSEDWEDAIVPHNLRVPVVPRAVVYATATEQIQAAVKCAVESEIRVSAKSGGHSYASMGLGGEDGSLVIQLDHWHDVTLRDDNTAVVSAGTRLGVVALELYAQGKRGISHGTCPSVGVGGHVVHGGYGFSSHTHGLALDAVVGANVVLADGSLVHASETENTDLFWALRGGGSSFGIVAEFEFETFDVSHNFSYFSIDSDISQETAEEATASLLAFQDALEEGLMDRKLNMRLSLGRPKVTLEAVYHGAKEDGRKALELFDDILGLNWSSNRTRANEADWLTMLESWTYGDPLNITYPYEGHDNAYTSSLVTRHIPEDAMASFMTYWKGVGQDRETPNWWLQMDVHGDANSRISEVDADSTAYSHRDKLWLFQFSSPLNPLRPDPEAAFALVNGYMDSIKDHLGDGEWGRYANYIDSELSREDAQTQYWSDHLDKLQAIKAELDPTQVFYNPQSIDPAAVE